European Patent Specification EP 3 392 337 B1, published March 6, 2024. Title: Gene-modified non-human animal, fertilized egg and method for the selective and site-specifically modifying a target gene. Applicant: Japan Science and Technology Agency. The sequence listing filed with the application follows.

SEQUENCE LISTING (82 sequences)

SEQ ID NO: 1 - protein, 7 aa, Artificial Sequence
  Artificial Sequence
PKKKRKV

SEQ ID NO: 2 - protein, 16 aa, Artificial Sequence
  Artificial Sequence
KRPAATKKAGQAKKKK

SEQ ID NO: 3 - protein, 9 aa, Artificial Sequence
  Artificial Sequence
PAAKRVKLD

SEQ ID NO: 4 - protein, 11 aa, Artificial Sequence
  Artificial Sequence
RQRRNELKRSP

SEQ ID NO: 5 - protein, 38 aa, Artificial Sequence
  Artificial Sequence
NQSSNFGPMKGGNFGGRSSGPYGGGGQYFAKPRNQGGY

SEQ ID NO: 6 - protein, 42 aa, Artificial Sequence
  Artificial Sequence
RMRIZFKNKGKDTAELRRRRVEVSVELRKAKKDEQILKRRNV

SEQ ID NO: 7 - protein, 8 aa, Artificial Sequence
  Artificial Sequence
VSRKRPRP

SEQ ID NO: 8 - protein, 8 aa, Artificial Sequence
  Artificial Sequence
PPKKARED

SEQ ID NO: 9 - protein, 8 aa, Artificial Sequence
  Artificial Sequence
PQPKKKPL

SEQ ID NO: 10 - protein, 12 aa, Artificial Sequence
  Artificial Sequence
SALIKKKKKMAP

SEQ ID NO: 11 - protein, 5 aa, Artificial Sequence
  Artificial Sequence
DRLRR

SEQ ID NO: 12 - protein, 6 aa, Artificial Sequence
  Artificial Sequence
PKQKKR

SEQ ID NO: 13 - protein, 10 aa, Artificial Sequence
  Artificial Sequence
RKLKKKIKKL

SEQ ID NO: 14 - protein, 10 aa, Artificial Sequence
  Artificial Sequence
REKKKFLKRR

SEQ ID NO: 15 - protein, 20 aa, Artificial Sequence
  Artificial Sequence
KRKGDEVDGVDEVAKKKSKK

SEQ ID NO: 16 - protein, 17 aa, Artificial Sequence
  Artificial Sequence
RKCLQAGMNLEARKTKK

SEQ ID NO: 17 - DNA, 4299 bp, Artificial Sequence
  Artificial Sequence
atgggacctaagaaaaagaggaaggtggccgccgctgactacaaggatgacgacgataaatctagactggaacccggcgagaagccatacaaatgcccagagtgtggtaaatctttctctcagtctggtgctctgaccagacaccagcggacccacactagagacaagaaatactctattggactggatatcggcacaaacagcgtcggctgggccgtcattacggacgagtacaaggtgccgagcaaaaaattcaaagttctgggcaataccgatcgccacagcataaagaagaacctcattggcgccctcctgttcgactccggggagacggccgaagccacgcggctcaaaagaacagcacggcgcagatatacccgcagaaagaatcggatctgctacctgcaggagatctttagtaatgagatggctaaggtggatgactctttcttccataggctggaggagtcctttttggtggaggaggataaaaagcacgagcgccacccaatctttggcaatatcgtggacgaggtggcgtaccatgaaaagtacccaaccatatatcatctgaggaagaagcttgtagacagtactgataaggctgacttgcggttgatctatctcgcgctggcgcatatgatcaaatttcggggacacttcctcatcgagggggacctgaacccagacaacagcgatgtcgacaaactctttatccaactggttcagacttacaatcagcttttcgaagagaacccgatcaacgcatccggagttgacgccaaagcaatcctgagcgctaggctgtccaaatcccggcggctcgaaaacctcatcgcacagctccctggggagaagaagaacggcctgtttggtaatcttatcgccctgtcactcgggctgacccccaactttaaatctaacttcgacctggccgaagatgccaagcttcaactgagcaaagacacctacgatgatgatctcgacaatctgctggcccagatcggcgaccagtacgcagacctttttttggcggcaaagaacctgtcagacgccattctgctgagtgatattctgcgagtgaacacggagatcaccaaagctccgctgagcgctagtatgatcaagcgctatgatgagcaccaccaagacttgactttgctgaaggcccttgtcagacagcaactgcctgagaagtacaaggaaattttcttcgatcagtctaaaaatggctacgccggatacattgacggcggagcaagccaggaggaattttacaaatttattaagcccatcttggaaaaaatggacggcaccgaggagctgctggtaaagcttaacagagaagatctgttgcgcaaacagcgcactttcgacaatggaagcatcccccaccagattcacctgggcgaactgcacgctatcctcaggcggcaagaggatttctacccctttttgaaagataacagggaaaagattgagaaaatcctcacatttcggataccctactatgtaggccccctcgcccggggaaattccagattcgcgtggatgactcgcaaatcagaagagaccatcactccctggaacttcgaggaagtcgtggataagggggcctctgcccagtccttcatcgaaaggatgactaactttgataaaaatctgcctaacgaaaaggtgcttcctaaacactctctgctgtacgagtacttcacagtttataacgagctcaccaaggtcaaatacgtcacagaagggatgagaaagccagcattcctgtctggagagcagaagaaagctatcgtggacctcctcttcaagacgaaccggaaagttaccgtgaaacagctcaaagaagactatttcaaaaagattgaatgtttcgactctgttgaaatcagcggagtggaggatcgcttcaacgcatccctgggaacgtatcacgatctcctgaaaatcattaaagacaaggacttcctggacaatgaggagaacgaggacattcttgaggacattgtcctcacccttacgttgtttgaagatagggagatgattgaagaacgcttgaaaacttacgctcatctcttcgacgacaaagtcatgaaacagctcaagaggcgccgatatacaggatgggggcggctgtcaagaaaactgatcaatgggatccgagacaagcagagtggaaagacaatcctggattttcttaagtccgatggatttgccaaccggaacttcatgcagttgatccatgatgactctctcacctttaaggaggacatccagaaagcacaagtttctggccagggggacagtcttcacgagcacatcgctaatcttgcaggtagcccagctatcaaaaagggaatactgcagaccgttaaggtcgtggatgaactcgtcaaagtaatgggaaggcataagcccgagaatatcgttatcgagatggcccgagagaaccaaactacccagaagggacagaagaacagtagggaaaggatgaagaggattgaagagggtataaaagaactggggtcccaaatccttaaggaacacccagttgaaaacacccagcttcagaatgagaagctctacctgtactacctgcagaacggcagggacatgtacgtggatcaggaactggacatcaatcggctctccgactacgacgtggatcatatcgtgccccagtcttttctcaaagatgattctattgataataaagtgttgacaagatccgataaaaatagagggaagagtgataacgtcccctcagaagaagttgtcaagaaaatgaaaaattattggcggcagctgctgaacgccaaactgatcacacaacggaagttcgataatctgactaaggctgaacgaggtggcctgtctgagttggataaagccggcttcatcaaaaggcagcttgttgagacacgccagatcaccaagcacgtggcccaaattctcgattcacgcatgaacaccaagtacgatgaaaatgacaaactgattcgagaggtgaaagttattactctgaagtctaagctggtctcagatttcagaaaggactttcagttttataaggtgagagagatcaacaattaccaccatgcgcatgatgcctacctgaatgcagtggtaggcactgcacttatcaaaaaatatcccaagcttgaatctgaatttgtttacggagactataaagtgtacgatgttaggaaaatgatcgcaaagtctgagcaggaaataggcaaggccaccgctaagtacttcttttacagcaatattatgaattttttcaagaccgagattacactggccaatggagagattcggaagcgaccacttatcgaaacaaacggagaaacaggagaaatcgtgtgggacaagggtagggatttcgcgacagtccggaaggtcctgtccatgccgcaggtgaacatcgttaaaaagaccgaagtacagaccggaggcttctccaaggaaagtatcctcccgaaaaggaacagcgacaagctgatcgcacgcaaaaaagattgggaccccaagaaatacggcggattcgattctcctacagtcgcttacagtgtactggttgtggccaaagtggagaaagggaagtctaaaaaactcaaaagcgtcaaggaactgctgggcatcacaatcatggagcgatcaagcttcgaaaaaaaccccatcgactttctcgaggcgaaaggatataaagaggtcaaaaaagacctcatcattaagcttcccaagtactctctctttgagcttgaaaacggccggaaacgaatgctcgctagtgcgggcgagctgcagaaaggtaacgagctggcactgccctctaaatacgttaatttcttgtatctggccagccactatgaaaagctcaaagggtctcccgaagataatgagcagaagcagctgttcgtggaacaacacaaacactaccttgatgagatcatcgagcaaataagcgaattctccaaaagagtgatcctcgccgacgctaacctcgataaggtgctttctgcttacaataagcacagggataagcccatcagggagcaggcagaaaacattatccacttgtttactctgaccaacttgggcgcgcctgcagccttcaagtacttcgacaccaccatagacagaaagcggtacacctctacaaaggaggtcctggacgccacactgattcatcagtcaattacggggctctatgaaacaagaatcgacctctctcagctcggtggagacagcagggctgaccccaagaagaagaggaaggtgtga

SEQ ID NO: 18 - DNA, 23 bp, Artificial Sequence
  Artificial Sequence
cgcagatgacagggtaaggaagg

SEQ ID NO: 19 - DNA, 23 bp, Artificial Sequence
  Artificial Sequence
atatgtattcgatcccacgttgg

SEQ ID NO: 20 - DNA, 23 bp, Artificial Sequence
  Artificial Sequence
atgtgatccgttggcaacttagg

SEQ ID NO: 21 - DNA, 23 bp, Artificial Sequence
  Artificial Sequence
gcgcgtcgtaccgtatggactgg

SEQ ID NO: 22 - DNA, 23 bp, Artificial Sequence
  Artificial Sequence
gagaaaataatgaatgtcaaagg

SEQ ID NO: 23 - DNA, 23 bp, Artificial Sequence
  Artificial Sequence
gggactgcgggtcggcatgacgg

SEQ ID NO: 24 - DNA, 23 bp, Artificial Sequence
  Artificial Sequence
ggctgccagacaacgtgccgggg

SEQ ID NO: 25 - DNA, 23 bp, Artificial Sequence
  Artificial Sequence
ggtcagcacccgcgtgggcatgg

SEQ ID NO: 26 - DNA, 23 bp, Artificial Sequence
  Artificial Sequence
gctctgcttgccatggccccggg

SEQ ID NO: 27 - DNA, 23 bp, Artificial Sequence
  Artificial Sequence
ggtgagcaccgtgtcgggcccgg

SEQ ID NO: 28 - DNA, 20 bp, Artificial Sequence
  Artificial Sequence
cggtgaagggtgttgtgtga

SEQ ID NO: 29 - DNA, 21 bp, Artificial Sequence
  Artificial Sequence
acacagtcatcaagcacaagc

SEQ ID NO: 30 - DNA, 24 bp, Artificial Sequence
  Artificial Sequence
ctaacgcctgctggtggtcacagt

SEQ ID NO: 31 - DNA, 20 bp, Artificial Sequence
  Artificial Sequence
tgtctagcccctgcttctct

SEQ ID NO: 32 - DNA, 25 bp, Artificial Sequence
  Artificial Sequence
gctctagagcctctgctaaccatgt

SEQ ID NO: 33 - DNA, 32 bp, Artificial Sequence
  Artificial Sequence
gcggaactccatatatgggctatgaactaatg

SEQ ID NO: 34 - DNA, 21 bp, Artificial Sequence
  Artificial Sequence
cgccgtgctgttcttttgagc

SEQ ID NO: 35 - DNA, 28 bp, Artificial Sequence
  Artificial Sequence
gccaccatggacaagaagtactccattg

SEQ ID NO: 36 - DNA, 28 bp, Artificial Sequence
  Artificial Sequence
ccatcgattcacaccttcctcttcttct

SEQ ID NO: 37 - DNA, 24 bp, Artificial Sequence
  Artificial Sequence
aagcgaattctccaaaagagtgat

SEQ ID NO: 38 - DNA, 20 bp, Artificial Sequence
  Artificial Sequence
agagtttgctgaggcaggtc

SEQ ID NO: 39 - DNA, 20 bp, Artificial Sequence
  Artificial Sequence
ccagcccatgtctcttccta

SEQ ID NO: 40 - DNA, 20 bp, Artificial Sequence
  Artificial Sequence
tggtgtggctgtagtccttc

SEQ ID NO: 41 - DNA, 20 bp, Artificial Sequence
  Artificial Sequence
caagtcaaaggggcctccac

SEQ ID NO: 42 - DNA, 21 bp, Artificial Sequence
  Artificial Sequence
tcaaccacacagctgtttctc

SEQ ID NO: 43 - DNA, 22 bp, Artificial Sequence
  Artificial Sequence
ctggcaccagtcacagggaatg

SEQ ID NO: 44 - DNA, 21 bp, Artificial Sequence
  Artificial Sequence
gttgttataatcttctaacag

SEQ ID NO: 45 - DNA, 21 bp, Artificial Sequence
  Artificial Sequence
ctgggtggaacaattgatcgt

SEQ ID NO: 46 - DNA, 18 bp, Artificial Sequence
  Artificial Sequence
tgagccattgctgaggcg

SEQ ID NO: 47 - DNA, 18 bp, Artificial Sequence
  Artificial Sequence
cgcgcctgatccttcctg

SEQ ID NO: 48 - DNA, 25 bp, Artificial Sequence
  Artificial Sequence
tgttggatacaggccagactttgtt

SEQ ID NO: 49 - DNA, 25 bp, Artificial Sequence
  Artificial Sequence
tcttaggctttgtatttggcttttc

SEQ ID NO: 50 - DNA, 20 bp, Artificial Sequence
  Artificial Sequence
acgcaggtaccaaccaatct

SEQ ID NO: 51 - DNA, 20 bp, Artificial Sequence
  Artificial Sequence
cccgggttcttcccttatgt

SEQ ID NO: 52 - DNA, 20 bp, Artificial Sequence
  Artificial Sequence
ggtacgcgctctcttaggtt

SEQ ID NO: 53 - DNA, 20 bp, Artificial Sequence
  Artificial Sequence
gcgtgtttcagatcgtctcc

SEQ ID NO: 54 - DNA, 20 bp, Artificial Sequence
  Artificial Sequence
gtcagagcgaggtgctgagt

SEQ ID NO: 55 - DNA, 23 bp, Artificial Sequence
  Artificial Sequence
cccatcaccactctactgtcttg

SEQ ID NO: 56 - DNA, 19 bp, Artificial Sequence
  Artificial Sequence
gcactggtggtctggagga

SEQ ID NO: 57 - DNA, 21 bp, Artificial Sequence
  Artificial Sequence
ccctcatcacctgggatacct

SEQ ID NO: 58 - DNA, 19 bp, Artificial Sequence
  Artificial Sequence
tgtgcctccctccgctgtt

SEQ ID NO: 59 - DNA, 21 bp, Artificial Sequence
  Artificial Sequence
ttactcctccacaccacaaga

SEQ ID NO: 60 - DNA, 18 bp, Artificial Sequence
  Artificial Sequence
ccgagctggaagcgagag

SEQ ID NO: 61 - DNA, 18 bp, Artificial Sequence
  Artificial Sequence
gacctctccgtccggtct

SEQ ID NO: 62 - DNA, 29 bp, Artificial Sequence
  Artificial Sequence
tcgaattcatcttagttggccatgaagac

SEQ ID NO: 63 - DNA, 31 bp, Artificial Sequence
  Artificial Sequence
tcgaattcacagcagccgatcagtgtgcttg

SEQ ID NO: 64 - DNA, 25 bp, Artificial Sequence
  Artificial Sequence
gtggctgaatgagactggtgtcgac

SEQ ID NO: 65 - DNA, 61 bp, Artificial Sequence
  Artificial Sequence
cgaagagtaaccgttgctaggagagaccgtggctgaatgagactggtgtcgacactagtgg

SEQ ID NO: 66 - DNA, 44 bp, Artificial Sequence
  Artificial Sequence
ccactagtgtcgacaccagtctctaattttttttttcaaaaaaa

SEQ ID NO: 67 - DNA, 25 bp, Artificial Sequence
  Artificial Sequence
tatatctgttttccaaccccagctc

SEQ ID NO: 68 - DNA, 25 bp, Artificial Sequence
  Artificial Sequence
tggggtacacgtagaccttttatga

SEQ ID NO: 69 - DNA, 26 bp, Artificial Sequence
  Artificial Sequence
tctctggctgaattgttttacacagg

SEQ ID NO: 70 - DNA, 23 bp, Artificial Sequence
  Artificial Sequence
aaagcagtcagcgaacctttttg

SEQ ID NO: 71 - DNA, 23 bp, Artificial Sequence
  Artificial Sequence
atgtctcgccagtccagtgtgtc

SEQ ID NO: 72 - DNA, 23 bp, Artificial Sequence
  Artificial Sequence
caccaccaaaaccaaatccactg

SEQ ID NO: 73 - DNA, 23 bp, Artificial Sequence
  Artificial Sequence
actcagacgtcttcgcacctgtc

SEQ ID NO: 74 - DNA, 23 bp, Artificial Sequence
  Artificial Sequence
cgccacatagtcggagttgtaga

SEQ ID NO: 75 - DNA, 23 bp, Artificial Sequence
  Artificial Sequence
cacctctgcagatgagggaagtg

SEQ ID NO: 76 - DNA, 23 bp, Artificial Sequence
  Artificial Sequence
gggcatcacctcgcagcttatag

SEQ ID NO: 77 - DNA, 22 bp, Artificial Sequence
  Artificial Sequence
cgcctttgacatgaaccaagtg

SEQ ID NO: 78 - DNA, 23 bp, Artificial Sequence
  Artificial Sequence
actcactgtagcctcgggacctc

SEQ ID NO: 79 - DNA, 44 bp, Artificial Sequence
  Artificial Sequence
cccgtaatccccagaccgtccatgcccacgcgggtgctgaccat

SEQ ID NO: 80 - DNA, 1067 bp, Artificial Sequence
  Artificial Sequence
tgtacaaactgcgccgcagccctgcgcgcgaagctcctggcccgcgaggggtgcggtcggcccgtcggaggcgggacctcgtgggccttctttcctactggctaccctctggccctggggccttgccattggccacaacgctgccagtccggtgagctggccctgcctccccggagttgggtgaaatagaggcgggcgtcaagtgtcagtagtcgcggggcaggtacgcgctctcttaggttgctggtggagcttgggggtggcgggagcgggttccggcgagagggtgagcgagcgctggggcggggcgggagaaagtggctgcccgaggacctcggcggtgacgcgtggccgagcccaggagccccgatctccgtgcccgccttcgtgagcgtctggctgccggcccaggggtcccccgccgcggccccccgccgagtccgccgtcccgtgccagcccgagcgaggtgggatcgcgatcgctccgtgtcccgctcccgtaatccccagaccggccatggactacaaagaccatgacggtgattataaagatcatgacatcgattacaaggatgacgatgacaagggaggatacccctacgacgtgcccgactacgccggaggacccacccgggtgctgaccatgagcgcccgcctgggaccactgccccagccgccggccgcgcaggacgagcccgtgttcgcgcagctcaagccggtgctgggcgctgcgaacccggcccgcgacgcggcgctcttctccggagacgatctgaaacacgcgcaccaccacccgcctgcgccgccgccagccgctggcccgcgactgccctcggaggagctggtccaggtaagcagagcggccggcctcccttccccggctcgggcgtgtcccgccgctacgaggcgcgggcgacaggggccgctccagactgggacgcgcgggaacgggtgcccgggtggacagccccgccctgcgctcccagacggggcgccggggagtggatgggggagcagggcgggggcccacccggatctgtccagaggagctaaagagaggcggccgc

SEQ ID NO: 81 - DNA, 30 bp, Artificial Sequence
  Artificial Sequence
ctgcaggaattcgccaccatgggacctaag

SEQ ID NO: 82 - DNA, 31 bp, Artificial Sequence
  Artificial Sequence
gctgtttgtgccgatagccagtccaatagag